European Patent Specification EP 3 959 208 B1, published July 5, 2023. Title: Cyclen based compounds, coordination compounds, peptides, pharmaceutical preparation, and use thereof. Applicant: Ustav organicke chemie a biochemie AV CR, v.v.i. The sequence listing filed with the application follows.

SEQUENCE LISTING (5 sequences)

SEQ ID NO: 1 - protein, 5 aa, artificial
  Pentapeptide synthesised in Example 28.
  (12) (1)..(1): (2S,3S,4S)-1-(((9H-fluoren-9-yl)methoxy)carbonyl)-4-acetoxy-3-(4, 7,10-tris(2-methoxy-2-oxoethyl)-1,4,7,10-tetraazacyclododecan-1-y l)pyrrolidine-2-carboxylic acid
  (Gd-6) (4)..(4): Gd(III) complex of 2,2',2''-(10-((2S,3S,4S)-2-carboxy-4-hydroxypyrrolidin-3-yl)-1,4, 7,10-tetraazacyclododecane-1,4,7-triyl)triacetic acid
XGFXG

SEQ ID NO: 2 - protein, 5 aa, artificial
  Pentapeptide synthesised in Example 29.
  (6) (1)..(1): 2,2',2''-(10-((2S,3S,4S)-(2-carboxy-4-hydroxypyrrolidin-3-yl)-1,4 ,7,10-tetraazacyclododecane-1,4,7-triyl)triacetic acid
  (Gd-6) (4)..(4): Gd(III) complex of 2,2',2''-(10-((2S,3S,4S)-2-carboxy-4-hydroxypyrrolidin-3-yl)-1,4, 7,10-tetraazacyclododecane-1,4,7-triyl)triacetic acid
XGFXG

SEQ ID NO: 3 - protein, 5 aa, artificial
  Pentapeptide synthesised in Example 30.
  (Lu-6) (1)..(1): Lu(III) complex of 2,2',2''-(10-((2S,3S,4S)-2-carboxy-4-hydroxypyrrolidin-3-yl)-1,4, 7,10-tetraazacyclododecane-1,4,7-triyl)triacetic acid
  (Gd-6) (4)..(4): Gd(III) complex of 2,2',2''-(10-((2S,3S,4S)-2-carboxy-4-hydroxypyrrolidin-3-yl)-1,4, 7,10-tetraazacyclododecane-1,4,7-triyl)triacetic acid
XGFXG

SEQ ID NO: 4 - protein, 4 aa, artificial
  Tetrapeptide synthesised in Example 31.
  (Gd-6) (3)..(3): Gd(III) complex of 2,2',2''-(10-((2S,3S,4S)-2-carboxy-4-hydroxypyrrolidin-3-yl)-1,4, 7,10-tetraazacyclododecane-1,4,7-triyl)triacetic acid
GFXG

SEQ ID NO: 5 - protein, 4 aa, artificial
  Tetrapeptide synthesised in Example 32.
  (Lu-6) (3)..(3): Lu(III) complex of 2,2',2''-(10-((2S,3S,4S)-2-carboxy-4-hydroxypyrrolidin-3-yl)-1,4, 7,10-tetraazacyclododecane-1,4,7-triyl)triacetic acid
GFXG